European Patent Application EP 4 786 002 A2, published August 5, 2026. Title: VACCINE COMPRISING IMMUNOGENIC FUSION PROTEINS. Applicant: MinervaX ApS. Application EP. The sequence listing filed with the application follows.

SEQUENCE LISTING (44 sequences)

SEQ ID NO: 1 - DNA, 525 bp, Streptococcus sp.
  source 1..525: mol_type = other DNA
atggctgaagtaatttcaggaagtgctgttacgttaaacacaaatatgactaaaaatgttcagaatggtagagcatatatagatttatatgatgtgaaaaatgggaaaatagatccattacaattaattacgttaaattcacctgatttaaaagctcagtatgtcattaggcaaggcggcaattatttcacacaaccttctgaattgactactgttggtgcagctagtattaattatacagtattgaagacagatggaagtcctcatacgaagcctgatggacaagtggatattataaacgtttcattgactatttacaattcttcagctttgagagataaaatagatgaagttaaaaagaaagcggaagaccctaaatgggacgagggaagtcgcgataaagttttgataagtttagatgatatcaaaacagatattgataataatcctaagacgcaatcagacattgccaataaaataactgaagttactaatttagaaaaaatactagtacctcgaatccca

SEQ ID NO: 2 - RNA, 525 nt, Streptococcus sp.
  source 1..525: mol_type = other RNA
atggctgaagtaatttcaggaagtgctgttacgttaaacacaaatatgactaaaaatgttcagaatggtagagcatatatagatttatatgatgtgaaaaatgggaaaatagatccattacaattaattacgttaaattcacctgatttaaaagctcagtatgtcattaggcaaggcggcaattatttcacacaaccttctgaattgactactgttggtgcagctagtattaattatacagtattgaagacagatggaagtcctcatacgaagcctgatggacaagtggatattataaacgtttcattgactatttacaattcttcagctttgagagataaaatagatgaagttaaaaagaaagcggaagaccctaaatgggacgagggaagtcgcgataaagttttgataagtttagatgatatcaaaacagatattgataataatcctaagacgcaatcagacattgccaataaaataactgaagttactaatttagaaaaaatactagtacctcgaatccca

SEQ ID NO: 3 - DNA, 525 bp, Streptococcus sp.
  source 1..525: mol_type = other DNA
atggccgaagttattagcggtagcgcagttaccctgaataccaatatgaccaaaaatgtgcagaatggccgtgcctatattgatctgtatgatgtgaaaaatggcaaaatcgatccgctgcagctgattaccctgaattctccggatctgaaagcacagtatgttattcgtcagggtggtaactattttacccagccgagcgaactgaccaccgttggtgcagcaagcattaactataccgttctgaaaaccgatggtagtccgcataccaaaccggatggtcaggttgatattatcaatgttagcctgaccatctataatagcagcgcactgcgtgataaaattgatgaagtgaaaaagaaagccgaagatccgaaatgggatgaaggtagccgtgataaagttctgattagcctggatgatatcaaaaccgatattgataacaacccgaaaacccagagcgatattgcaaacaaaattaccgaagtgaccaatctggaaaaaattctggttccgcgtattccg

SEQ ID NO: 4 - RNA, 525 nt, Streptococcus sp.
  source 1..525: mol_type = other RNA
atggccgaagttattagcggtagcgcagttaccctgaataccaatatgaccaaaaatgtgcagaatggccgtgcctatattgatctgtatgatgtgaaaaatggcaaaatcgatccgctgcagctgattaccctgaattctccggatctgaaagcacagtatgttattcgtcagggtggtaactattttacccagccgagcgaactgaccaccgttggtgcagcaagcattaactataccgttctgaaaaccgatggtagtccgcataccaaaccggatggtcaggttgatattatcaatgttagcctgaccatctataatagcagcgcactgcgtgataaaattgatgaagtgaaaaagaaagccgaagatccgaaatgggatgaaggtagccgtgataaagttctgattagcctggatgatatcaaaaccgatattgataacaacccgaaaacccagagcgatattgcaaacaaaattaccgaagtgaccaatctggaaaaaattctggttccgcgtattccg

SEQ ID NO: 5 - DNA, 525 bp, Streptococcus sp.
  source 1..525: mol_type = other DNA
atggccgaagtgatctccggctctgctgtgaccctgaacaccaacatgaccaagaacgtgcagaacggcagagcctacatcgacctgtacgatgtgaagaacggcaagatcgaccctctgcagctgatcaccctgaactctcccgatctgaaggcccagtacgtgatcagacaaggcggcaactacttcacccagccttccgagctgaccaccgtgggagccgcctctatcaattacaccgtgctgaaaaccgacggctcccctcacaccaagcctgatggacaggtggacatcatcaacgtgtccctgaccatctacaacagcagcgccctgcgggacaagatcgatgaagtgaagaagaaggccgaggatcccaagtgggacgagggctctagagacaaggtgctgatctccctggacgacatcaagaccgacatcgacaacaaccccaagacacagtccgatatcgccaacaagatcaccgaagtgaccaacctcgagaagatcctggtgcctcggatcccc

SEQ ID NO: 6 - RNA, 525 nt, Streptococcus sp.
  source 1..525: mol_type = other RNA
atggccgaagtgatctccggctctgctgtgaccctgaacaccaacatgaccaagaacgtgcagaacggcagagcctacatcgacctgtacgatgtgaagaacggcaagatcgaccctctgcagctgatcaccctgaactctcccgatctgaaggcccagtacgtgatcagacaaggcggcaactacttcacccagccttccgagctgaccaccgtgggagccgcctctatcaattacaccgtgctgaaaaccgacggctcccctcacaccaagcctgatggacaggtggacatcatcaacgtgtccctgaccatctacaacagcagcgccctgcgggacaagatcgatgaagtgaagaagaaggccgaggatcccaagtgggacgagggctctagagacaaggtgctgatctccctggacgacatcaagaccgacatcgacaacaaccccaagacacagtccgatatcgccaacaagatcaccgaagtgaccaacctcgagaagatcctggtgcctcggatcccc

SEQ ID NO: 7 - protein, 175 aa, Streptococcus sp.
MAEVISGSAVTLNTNMTKNVQNGRAYIDLYDVKNGKIDPLQLITLNSPDLKAQYVIRQGGNYFTQPSELTTVGAASINYTVLKTDGSPHTKPDGQVDIINVSLTIYNSSALRDKIDEVKKKAEDPKWDEGSRDKVLISLDDIKTDIDNNPKTQSDIANKITEVTNLEKILVPRIP

SEQ ID NO: 8 - DNA, 516 bp, Streptococcus sp.
  source 1..516: mol_type = other DNA
tctacaattccagggagtgcagcgaccttaaatacaagcatcactaaaaatatacaaaacggaaatgcttacatagatttatatgatgtaaaattaggtaaaatagatccattacaattaattgttttagaacaaggttttacagcaaagtatgtttttagacaaggtactaaatactatggggatgtttctcagttgcagagtacaggaagggctagtcttacctataatatatttggtgaagatggactaccacatgtaaagactgatggacaaattgatatagttagtgttgctttaactatttatgattcaacaaccttgagggataagattgaagaagttagaacgaatgcaaacgatcctaagtggacggaagaaagtcgtactgaggttttaacaggattagatacaattaagacagatattgataataatcctaagacgcaaacagatattgatagtaaaattgttgaggttaatgaattagagaaattgttagtattgtcataataa

SEQ ID NO: 9 - RNA, 516 nt, Streptococcus sp.
  source 1..516: mol_type = other RNA
tctacaattccagggagtgcagcgaccttaaatacaagcatcactaaaaatatacaaaacggaaatgcttacatagatttatatgatgtaaaattaggtaaaatagatccattacaattaattgttttagaacaaggttttacagcaaagtatgtttttagacaaggtactaaatactatggggatgtttctcagttgcagagtacaggaagggctagtcttacctataatatatttggtgaagatggactaccacatgtaaagactgatggacaaattgatatagttagtgttgctttaactatttatgattcaacaaccttgagggataagattgaagaagttagaacgaatgcaaacgatcctaagtggacggaagaaagtcgtactgaggttttaacaggattagatacaattaagacagatattgataataatcctaagacgcaaacagatattgatagtaaaattgttgaggttaatgaattagagaaattgttagtattgtcataataa

SEQ ID NO: 10 - DNA, 516 bp, Streptococcus sp.
  source 1..516: mol_type = other DNA
agcaccattccgggtagcgcagcaacactgaatacaagcattaccaaaaacattcagaacggcaacgcatatatcgatctgtacgacgttaaactgggtaaaattgatcctctgcaactgatcgttctggaacagggttttaccgcaaaatatgtgtttcgtcagggcaccaaatactatggtgatgttagccagctgcagagcaccggtcgtgcaagcctgacctataacatttttggtgaagatggtctgccgcatgttaaaaccgatggccagattgatatcgttagcgttgcactgacgatttatgatagcaccaccctgcgcgataaaatcgaagaagttcgtaccaacgcaaacgatcctaaatggaccgaagaaagccgtaccgaagttctgaccggtctggataccattaaaacggatatcgacaataatcctaaaacgcagacagatattgatagcaaaattgtggaagtgaatgaactggaaaaactgctggttctgagctaataa

SEQ ID NO: 11 - RNA, 516 nt, Streptococcus sp.
  source 1..516: mol_type = other RNA
agcaccattccgggtagcgcagcaacactgaatacaagcattaccaaaaacattcagaacggcaacgcatatatcgatctgtacgacgttaaactgggtaaaattgatcctctgcaactgatcgttctggaacagggttttaccgcaaaatatgtgtttcgtcagggcaccaaatactatggtgatgttagccagctgcagagcaccggtcgtgcaagcctgacctataacatttttggtgaagatggtctgccgcatgttaaaaccgatggccagattgatatcgttagcgttgcactgacgatttatgatagcaccaccctgcgcgataaaatcgaagaagttcgtaccaacgcaaacgatcctaaatggaccgaagaaagccgtaccgaagttctgaccggtctggataccattaaaacggatatcgacaataatcctaaaacgcagacagatattgatagcaaaattgtggaagtgaatgaactggaaaaactgctggttctgagctaataa

SEQ ID NO: 12 - DNA, 516 bp, Streptococcus sp.
  source 1..516: mol_type = other DNA
agcacaatccctggatctgccgccacactgaacacctctatcaccaagaacatccagaatgggaacgcttacatcgatctctacgacgtcaagctgggcaagattgatcccctccagctcatcgtgctggaacagggcttcaccgccaaatacgtgttccggcagggcaccaagtactacggggatgtgtcacagctgcagtccaccggcagagcttccctgacctacaacatcttcggcgaggatggcctgcctcacgtgaaaacagatggccagatcgacatcgtgtctgtggctctgacaatctacgactccaccacactgcgcgataagattgaggaagtgcggaccaacgccaacgatcctaagtggaccgaggaatccagaaccgaggtgctgaccggcctggacaccattaagacagatattgataacaatcctaagactcagacagacatcgattccaagatcgtggaagtcaacgagctggaaaagctgctggtgctgtcctgatga

SEQ ID NO: 13 - RNA, 516 nt, Streptococcus sp.
  source 1..516: mol_type = other RNA
agcacaatccctggatctgccgccacactgaacacctctatcaccaagaacatccagaatgggaacgcttacatcgatctctacgacgtcaagctgggcaagattgatcccctccagctcatcgtgctggaacagggcttcaccgccaaatacgtgttccggcagggcaccaagtactacggggatgtgtcacagctgcagtccaccggcagagcttccctgacctacaacatcttcggcgaggatggcctgcctcacgtgaaaacagatggccagatcgacatcgtgtctgtggctctgacaatctacgactccaccacactgcgcgataagattgaggaagtgcggaccaacgccaacgatcctaagtggaccgaggaatccagaaccgaggtgctgaccggcctggacaccattaagacagatattgataacaatcctaagactcagacagacatcgattccaagatcgtggaagtcaacgagctggaaaagctgctggtgctgtcctgatga

SEQ ID NO: 14 - protein, 170 aa, Streptococcus sp.
STIPGSAATLNTSITKNIQNGNAYIDLYDVKLGKIDPLQLIVLEQGFTAKYVFRQGTKYYGDVSQLQSTGRASLTYNIFGEDGLPHVKTDGQIDIVSVALTIYDSTTLRDKIEEVRTNANDPKWTEESRTEVLTGLDTIKTDIDNNPKTQTDIDSKIVEVNELEKLLVLS

SEQ ID NO: 15 - DNA, 1047 bp, Streptococcus sp.
  source 1..1047: mol_type = other DNA
atggctgaagtaatttcaggaagtgctgttacgttaaacacaaatatgactaaaaatgttcagaatggtagagcatatatagatttatatgatgtgaaaaatgggaaaatagatccattacaattaattacgttaaattcacctgatttaaaagctcagtatgtcattaggcaaggcggcaattatttcacacaaccttctgaattgactactgttggtgcagctagtattaattatacagtattgaagacagatggaagtcctcatacgaagcctgatggacaagtggatattataaacgtttcattgactatttacaattcttcagctttgagagataaaatagatgaagttaaaaagaaagcggaagaccctaaatgggacgagggaagtcgcgataaagttttgataagtttagatgatatcaaaacagatattgataataatcctaagacgcaatcagacattgccaataaaataactgaagttactaatttagaaaaaatactagtacctcgaatcccagaattctctacaattccagggagtgcagcgaccttaaatacaagcatcactaaaaatatacaaaacggaaatgcttacatagatttatatgatgtaaaattaggtaaaatagatccattacaattaattgttttagaacaaggttttacagcaaagtatgtttttagacaaggtactaaatactatggggatgtttctcagttgcagagtacaggaagggctagtcttacctataatatatttggtgaagatggactaccacatgtaaagactgatggacaaattgatatagttagtgttgctttaactatttatgattcaacaaccttgagggataagattgaagaagttagaacgaatgcaaacgatcctaagtggacggaagaaagtcgtactgaggttttaacaggattagatacaattaagacagatattgataataatcctaagacgcaaacagatattgatagtaaaattgttgaggttaatgaattagagaaattgttagtattgtcataataa

SEQ ID NO: 16 - RNA, 1047 nt, Streptococcus sp.
  source 1..1047: mol_type = other RNA
atggctgaagtaatttcaggaagtgctgttacgttaaacacaaatatgactaaaaatgttcagaatggtagagcatatatagatttatatgatgtgaaaaatgggaaaatagatccattacaattaattacgttaaattcacctgatttaaaagctcagtatgtcattaggcaaggcggcaattatttcacacaaccttctgaattgactactgttggtgcagctagtattaattatacagtattgaagacagatggaagtcctcatacgaagcctgatggacaagtggatattataaacgtttcattgactatttacaattcttcagctttgagagataaaatagatgaagttaaaaagaaagcggaagaccctaaatgggacgagggaagtcgcgataaagttttgataagtttagatgatatcaaaacagatattgataataatcctaagacgcaatcagacattgccaataaaataactgaagttactaatttagaaaaaatactagtacctcgaatcccagaattctctacaattccagggagtgcagcgaccttaaatacaagcatcactaaaaatatacaaaacggaaatgcttacatagatttatatgatgtaaaattaggtaaaatagatccattacaattaattgttttagaacaaggttttacagcaaagtatgtttttagacaaggtactaaatactatggggatgtttctcagttgcagagtacaggaagggctagtcttacctataatatatttggtgaagatggactaccacatgtaaagactgatggacaaattgatatagttagtgttgctttaactatttatgattcaacaaccttgagggataagattgaagaagttagaacgaatgcaaacgatcctaagtggacggaagaaagtcgtactgaggttttaacaggattagatacaattaagacagatattgataataatcctaagacgcaaacagatattgatagtaaaattgttgaggttaatgaattagagaaattgttagtattgtcataataa

SEQ ID NO: 17 - DNA, 1047 bp, Streptococcus sp.
  source 1..1047: mol_type = other DNA
atggccgaagttattagcggtagcgcagttaccctgaataccaatatgaccaaaaatgtgcagaatggccgtgcctatattgatctgtatgatgtgaaaaatggcaaaatcgatccgctgcagctgattaccctgaattctccggatctgaaagcacagtatgttattcgtcagggtggtaactattttacccagccgagcgaactgaccaccgttggtgcagcaagcattaactataccgttctgaaaaccgatggtagtccgcataccaaaccggatggtcaggttgatattatcaatgttagcctgaccatctataatagcagcgcactgcgtgataaaattgatgaagtgaaaaagaaagccgaagatccgaaatgggatgaaggtagccgtgataaagttctgattagcctggatgatatcaaaaccgatattgataacaacccgaaaacccagagcgatattgcaaacaaaattaccgaagtgaccaatctggaaaaaattctggttccgcgtattccggaatttagcaccattccgggtagcgcagcaacactgaatacaagcattaccaaaaacattcagaacggcaacgcatatatcgatctgtacgacgttaaactgggtaaaattgatcctctgcaactgatcgttctggaacagggttttaccgcaaaatatgtgtttcgtcagggcaccaaatactatggtgatgttagccagctgcagagcaccggtcgtgcaagcctgacctataacatttttggtgaagatggtctgccgcatgttaaaaccgatggccagattgatatcgttagcgttgcactgacgatttatgatagcaccaccctgcgcgataaaatcgaagaagttcgtaccaacgcaaacgatcctaaatggaccgaagaaagccgtaccgaagttctgaccggtctggataccattaaaacggatatcgacaataatcctaaaacgcagacagatattgatagcaaaattgtggaagtgaatgaactggaaaaactgctggttctgagctaataa

SEQ ID NO: 18 - RNA, 1047 nt, Streptococcus sp.
  source 1..1047: mol_type = other RNA
atggccgaagttattagcggtagcgcagttaccctgaataccaatatgaccaaaaatgtgcagaatggccgtgcctatattgatctgtatgatgtgaaaaatggcaaaatcgatccgctgcagctgattaccctgaattctccggatctgaaagcacagtatgttattcgtcagggtggtaactattttacccagccgagcgaactgaccaccgttggtgcagcaagcattaactataccgttctgaaaaccgatggtagtccgcataccaaaccggatggtcaggttgatattatcaatgttagcctgaccatctataatagcagcgcactgcgtgataaaattgatgaagtgaaaaagaaagccgaagatccgaaatgggatgaaggtagccgtgataaagttctgattagcctggatgatatcaaaaccgatattgataacaacccgaaaacccagagcgatattgcaaacaaaattaccgaagtgaccaatctggaaaaaattctggttccgcgtattccggaatttagcaccattccgggtagcgcagcaacactgaatacaagcattaccaaaaacattcagaacggcaacgcatatatcgatctgtacgacgttaaactgggtaaaattgatcctctgcaactgatcgttctggaacagggttttaccgcaaaatatgtgtttcgtcagggcaccaaatactatggtgatgttagccagctgcagagcaccggtcgtgcaagcctgacctataacatttttggtgaagatggtctgccgcatgttaaaaccgatggccagattgatatcgttagcgttgcactgacgatttatgatagcaccaccctgcgcgataaaatcgaagaagttcgtaccaacgcaaacgatcctaaatggaccgaagaaagccgtaccgaagttctgaccggtctggataccattaaaacggatatcgacaataatcctaaaacgcagacagatattgatagcaaaattgtggaagtgaatgaactggaaaaactgctggttctgagctaataa

SEQ ID NO: 19 - DNA, 1047 bp, Streptococcus sp.
  source 1..1047: mol_type = other DNA
atggccgaagtgatctccggctctgctgtgaccctgaacaccaacatgaccaagaacgtgcagaacggcagagcctacatcgacctgtacgatgtgaagaacggcaagatcgaccctctgcagctgatcaccctgaactctcccgatctgaaggcccagtacgtgatcagacaaggcggcaactacttcacccagccttccgagctgaccaccgtgggagccgcctctatcaattacaccgtgctgaaaaccgacggctcccctcacaccaagcctgatggacaggtggacatcatcaacgtgtccctgaccatctacaacagcagcgccctgcgggacaagatcgatgaagtgaagaagaaggccgaggatcccaagtgggacgagggctctagagacaaggtgctgatctccctggacgacatcaagaccgacatcgacaacaaccccaagacacagtccgatatcgccaacaagatcaccgaagtgaccaacctcgagaagatcctggtgcctcggatccccgagttcagcacaatccctggatctgccgccacactgaacacctctatcaccaagaacatccagaatgggaacgcttacatcgatctctacgacgtcaagctgggcaagattgatcccctccagctcatcgtgctggaacagggcttcaccgccaaatacgtgttccggcagggcaccaagtactacggggatgtgtcacagctgcagtccaccggcagagcttccctgacctacaacatcttcggcgaggatggcctgcctcacgtgaaaacagatggccagatcgacatcgtgtctgtggctctgacaatctacgactccaccacactgcgcgataagattgaggaagtgcggaccaacgccaacgatcctaagtggaccgaggaatccagaaccgaggtgctgaccggcctggacaccattaagacagatattgataacaatcctaagactcagacagacatcgattccaagatcgtggaagtcaacgagctggaaaagctgctggtgctgtcctgatga

SEQ ID NO: 20 - RNA, 1047 nt, Streptococcus sp.
  source 1..1047: mol_type = other RNA
atggccgaagtgatctccggctctgctgtgaccctgaacaccaacatgaccaagaacgtgcagaacggcagagcctacatcgacctgtacgatgtgaagaacggcaagatcgaccctctgcagctgatcaccctgaactctcccgatctgaaggcccagtacgtgatcagacaaggcggcaactacttcacccagccttccgagctgaccaccgtgggagccgcctctatcaattacaccgtgctgaaaaccgacggctcccctcacaccaagcctgatggacaggtggacatcatcaacgtgtccctgaccatctacaacagcagcgccctgcgggacaagatcgatgaagtgaagaagaaggccgaggatcccaagtgggacgagggctctagagacaaggtgctgatctccctggacgacatcaagaccgacatcgacaacaaccccaagacacagtccgatatcgccaacaagatcaccgaagtgaccaacctcgagaagatcctggtgcctcggatccccgagttcagcacaatccctggatctgccgccacactgaacacctctatcaccaagaacatccagaatgggaacgcttacatcgatctctacgacgtcaagctgggcaagattgatcccctccagctcatcgtgctggaacagggcttcaccgccaaatacgtgttccggcagggcaccaagtactacggggatgtgtcacagctgcagtccaccggcagagcttccctgacctacaacatcttcggcgaggatggcctgcctcacgtgaaaacagatggccagatcgacatcgtgtctgtggctctgacaatctacgactccaccacactgcgcgataagattgaggaagtgcggaccaacgccaacgatcctaagtggaccgaggaatccagaaccgaggtgctgaccggcctggacaccattaagacagatattgataacaatcctaagactcagacagacatcgattccaagatcgtggaagtcaacgagctggaaaagctgctggtgctgtcctgatga

SEQ ID NO: 21 - protein, 347 aa, Streptococcus sp.
MAEVISGSAVTLNTNMTKNVQNGRAYIDLYDVKNGKIDPLQLITLNSPDLKAQYVIRQGGNYFTQPSELTTVGAASINYTVLKTDGSPHTKPDGQVDIINVSLTIYNSSALRDKIDEVKKKAEDPKWDEGSRDKVLISLDDIKTDIDNNPKTQSDIANKITEVTNLEKILVPRIPEFSTIPGSAATLNTSITKNIQNGNAYIDLYDVKLGKIDPLQLIVLEQGFTAKYVFRQGTKYYGDVSQLQSTGRASLTYNIFGEDGLPHVKTDGQIDIVSVALTIYDSTTLRDKIEEVRTNANDPKWTEESRTEVLTGLDTIKTDIDNNPKTQTDIDSKIVEVNELEKLLVLS

SEQ ID NO: 22 - DNA, 519 bp, Streptococcus sp.
  source 1..519: mol_type = other DNA
atggccgaagttattagcggtagcgcagcaaccctgaatagcgcactggttaaaaatgttagcggtggcaaagcctatatcgacatctatgatgtgaaaaacggcaaaattgatccgctgaatctgattgttctgcctccgagcaattatagcgccaactattatatcaaacagggtggtcgcattttcaccaatgttaatcagctgcagacaccgggtacagcaaccattacctataacattctggatgaaaatggcaacccgtataccaaaagtgatggccagattgatattgttagcctggttaccaccgtttatgataccaccgaactgcgcaataacatcaacaaagttattgagaatgccaacgacccgaaatggtcagatgatagccgtaaagatgttctgagcaaaatcgaggtgatcaaaaacgatattgataacaacccgaaaacccagagcgatatcgacaacaaaattgtggaagtgaacgagctggaaaaactgctggttctgccg

SEQ ID NO: 23 - RNA, 519 nt, Streptococcus sp.
  source 1..519: mol_type = other RNA
atggccgaagttattagcggtagcgcagcaaccctgaatagcgcactggttaaaaatgttagcggtggcaaagcctatatcgacatctatgatgtgaaaaacggcaaaattgatccgctgaatctgattgttctgcctccgagcaattatagcgccaactattatatcaaacagggtggtcgcattttcaccaatgttaatcagctgcagacaccgggtacagcaaccattacctataacattctggatgaaaatggcaacccgtataccaaaagtgatggccagattgatattgttagcctggttaccaccgtttatgataccaccgaactgcgcaataacatcaacaaagttattgagaatgccaacgacccgaaatggtcagatgatagccgtaaagatgttctgagcaaaatcgaggtgatcaaaaacgatattgataacaacccgaaaacccagagcgatatcgacaacaaaattgtggaagtgaacgagctggaaaaactgctggttctgccg

SEQ ID NO: 24 - DNA, 519 bp, Streptococcus sp.
  source 1..519: mol_type = other DNA
atggccgaagttattagcggtagcgcagcaaccctgaatagcgcactggttaaaaatgttagcggtggcaaagcctatatcgacatctatgatgtgaaaaacggcaaaattgatccgctgaatctgattgttctgaccccgagcaattatagcgccaactattatatcaaacagggtggtcgtattttcaccagcgttaatcagctgcagacaccgggtacagcaaccattacctataacattctggatgaaaatggcaacccgtataccaaaagtgatggccagattgatattgttagcctggttaccaccgtttatgataccaccgaactgcgcaataacatcaacaaagttattgagaatgccaacgacccgaaatggtcagatgatagccgtaaagatgttctgagcaaaatcgaggtgatcaaaaacgatattgataacaacccgaaaacccagagcgatatcgacaacaaaattgtggaagtgaacgagctggaaaaactgctggttctgccg

SEQ ID NO: 25 - RNA, 519 nt, Streptococcus sp.
  source 1..519: mol_type = other RNA
atggccgaagttattagcggtagcgcagcaaccctgaatagcgcactggttaaaaatgttagcggtggcaaagcctatatcgacatctatgatgtgaaaaacggcaaaattgatccgctgaatctgattgttctgaccccgagcaattatagcgccaactattatatcaaacagggtggtcgtattttcaccagcgttaatcagctgcagacaccgggtacagcaaccattacctataacattctggatgaaaatggcaacccgtataccaaaagtgatggccagattgatattgttagcctggttaccaccgtttatgataccaccgaactgcgcaataacatcaacaaagttattgagaatgccaacgacccgaaatggtcagatgatagccgtaaagatgttctgagcaaaatcgaggtgatcaaaaacgatattgataacaacccgaaaacccagagcgatatcgacaacaaaattgtggaagtgaacgagctggaaaaactgctggttctgccg

SEQ ID NO: 26 - DNA, 519 bp, Streptococcus sp.
  source 1..519: mol_type = other DNA
atggccgaagtgatctccggctctgctgctaccctgaactctgccctggtcaagaatgtgtctggcggcaaggcctacatcgacatctacgacgtgaagaacggcaagatcgaccctctgaacctgatcgtgctgaccccttccaactactccgccaactactacatcaagcaaggcggcagaatcttcacctccgtgaaccagctgcagacccctggcaccgctaccatcacctacaacatcctggacgagaatggcaacccctacaccaagtccgacggccagatcgatatcgtgtccctggtcaccaccgtgtacgacaccaccgagctgcggaacaacatcaacaaagtgatcgagaacgccaacgatcccaagtggagcgacgactctagaaaggacgtgctgtccaagatcgaagtcatcaagaacgacatcgacaacaaccccaagacacagtccgacattgataacaagatcgtggaagtgaacgagctggaaaagctgctggtgctgccc

SEQ ID NO: 27 - RNA, 519 nt, Streptococcus sp.
  source 1..519: mol_type = other RNA
atggccgaagtgatctccggctctgctgctaccctgaactctgccctggtcaagaatgtgtctggcggcaaggcctacatcgacatctacgacgtgaagaacggcaagatcgaccctctgaacctgatcgtgctgaccccttccaactactccgccaactactacatcaagcaaggcggcagaatcttcacctccgtgaaccagctgcagacccctggcaccgctaccatcacctacaacatcctggacgagaatggcaacccctacaccaagtccgacggccagatcgatatcgtgtccctggtcaccaccgtgtacgacaccaccgagctgcggaacaacatcaacaaagtgatcgagaacgccaacgatcccaagtggagcgacgactctagaaaggacgtgctgtccaagatcgaagtcatcaagaacgacatcgacaacaaccccaagacacagtccgacattgataacaagatcgtggaagtgaacgagctggaaaagctgctggtgctgccc

SEQ ID NO: 28 - protein, 173 aa, Streptococcus sp.
MAEVISGSAATLNSALVKNVSGGKAYIDIYDVKNGKIDPLNLIVLTPSNYSANYYIKQGGRIFTSVNQLQTPGTATITYNILDENGNPYTKSDGQIDIVSLVTTVYDTTELRNNINKVIENANDPKWSDDSRKDVLSKIEVIKNDIDNNPKTQSDIDNKIVEVNELEKLLVLP

SEQ ID NO: 29 - DNA, 522 bp, Streptococcus sp.
  source 1..522: mol_type = other DNA
agcaccattccgggttcagcagccacactgaataccagcattaccaaaaacattcagaatggcaacgcctacattgatctgtacgatgtaaaaaatggtctgatcgatccgcagaacctgatcgtgctgaatccgagcagctattcagccaattattatattaaacaaggcgcaaaatactatagcaacccgagcgaaattaccaccaccggtagcgccaccattacgtttaatatcctggacgaaaccggtaacccgcataaaaaagcagatggtcaaattgatatcgtgagcgttaacctgacgatttatgatagcacagccctgcgtaatcgtattgatgaagtgattaataacgcgaatgatcctaaatggtccgatggtagtcgtgatgaagtactgaccggtctggaaaaaatcaaaaaagacatcgacaataatccgaaaacgcagattgacattgacaataaaatcaacgaggtgaacgagatcgagaaactgctggtagttagcctgtaataa

SEQ ID NO: 30 - RNA, 522 nt, Streptococcus sp.
  source 1..522: mol_type = other RNA
agcaccattccgggttcagcagccacactgaataccagcattaccaaaaacattcagaatggcaacgcctacattgatctgtacgatgtaaaaaatggtctgatcgatccgcagaacctgatcgtgctgaatccgagcagctattcagccaattattatattaaacaaggcgcaaaatactatagcaacccgagcgaaattaccaccaccggtagcgccaccattacgtttaatatcctggacgaaaccggtaacccgcataaaaaagcagatggtcaaattgatatcgtgagcgttaacctgacgatttatgatagcacagccctgcgtaatcgtattgatgaagtgattaataacgcgaatgatcctaaatggtccgatggtagtcgtgatgaagtactgaccggtctggaaaaaatcaaaaaagacatcgacaataatccgaaaacgcagattgacattgacaataaaatcaacgaggtgaacgagatcgagaaactgctggtagttagcctgtaataa

SEQ ID NO: 31 - DNA, 522 bp, Streptococcus sp.; identical to SEQ ID NO: 29
  source 1..522: mol_type = other DNA

SEQ ID NO: 32 - RNA, 522 nt, Streptococcus sp.; identical to SEQ ID NO: 30
  source 1..522: mol_type = other RNA

SEQ ID NO: 33 - DNA, 522 bp, Streptococcus sp.
  source 1..522: mol_type = other DNA
agcacaatccctggatctgccgccacactgaacacctccatcaccaagaatatccagaacgggaacgcttacatcgacctgtatgatgtcaagaacgggctgatcgatccccagaatctgattgtgctcaacccctcctcctactctgctaattactatattaagcagggcgccaagtactactctaacccctccgagatcaccaccaccggctccgccaccatcacattcaatattctggatgagacaggcaaccctcacaagaaggctgacggacagattgacattgtgtctgtgaacctgaccatctacgattccaccgctctgcggaaccggatcgatgaagtgatcaacaacgctaatgaccctaagtggagtgacggctccagagatgaggtgctgaccggcctggaaaagatcaagaaggatatcgataacaatcctaaaactcagatcgatattgacaacaagatcaacgaagtcaacgagatcgagaagctcctggtcgtgtctctgtgatga

SEQ ID NO: 34 - RNA, 522 nt, Streptococcus sp.
  source 1..522: mol_type = other RNA
agcacaatccctggatctgccgccacactgaacacctccatcaccaagaatatccagaacgggaacgcttacatcgacctgtatgatgtcaagaacgggctgatcgatccccagaatctgattgtgctcaacccctcctcctactctgctaattactatattaagcagggcgccaagtactactctaacccctccgagatcaccaccaccggctccgccaccatcacattcaatattctggatgagacaggcaaccctcacaagaaggctgacggacagattgacattgtgtctgtgaacctgaccatctacgattccaccgctctgcggaaccggatcgatgaagtgatcaacaacgctaatgaccctaagtggagtgacggctccagagatgaggtgctgaccggcctggaaaagatcaagaaggatatcgataacaatcctaaaactcagatcgatattgacaacaagatcaacgaagtcaacgagatcgagaagctcctggtcgtgtctctgtgatga

SEQ ID NO: 35 - protein, 172 aa, Streptococcus sp.
STIPGSAATLNTSITKNIQNGNAYIDLYDVKNGLIDPQNLIVLNPSSYSANYYIKQGAKYYSNPSEITTTGSATITFNILDETGNPHKKADGQIDIVSVNLTIYDSTALRNRIDEVINNANDPKWSDGSRDEVLTGLEKIKKDIDNNPKTQIDIDNKINEVNEIEKLLVVSL

SEQ ID NO: 36 - DNA, 1047 bp, Streptococcus sp.
  source 1..1047: mol_type = other DNA
atggccgaagttattagcggtagcgcagcaaccctgaatagcgcactggttaaaaatgttagcggtggcaaagcctatatcgacatctatgatgtgaaaaacggcaaaattgatccgctgaatctgattgttctgcctccgagcaattatagcgccaactattatatcaaacagggtggtcgcattttcaccaatgttaatcagctgcagacaccgggtacagcaaccattacctataacattctggatgaaaatggcaacccgtataccaaaagtgatggccagattgatattgttagcctggttaccaccgtttatgataccaccgaactgcgcaataacatcaacaaagttattgagaatgccaacgacccgaaatggtcagatgatagccgtaaagatgttctgagcaaaatcgaggtgatcaaaaacgatattgataacaacccgaaaacccagagcgatatcgacaacaaaattgtggaagtgaacgagctggaaaaactgctggttctgccggaatttagcaccattccgggttcagcagccacactgaataccagcattaccaaaaacattcagaatggcaacgcctacattgatctgtacgatgtaaaaaatggtctgatcgatccgcagaacctgatcgtgctgaatccgagcagctattcagccaattattatattaaacaaggcgcaaaatactatagcaacccgagcgaaattaccaccaccggtagcgccaccattacgtttaatatcctggacgaaaccggtaacccgcataaaaaagcagatggtcaaattgatatcgtgagcgttaacctgacgatttatgatagcacagccctgcgtaatcgtattgatgaagtgattaataacgcgaatgatcctaaatggtccgatggtagtcgtgatgaagtactgaccggtctggaaaaaatcaaaaaagacatcgacaataatccgaaaacgcagattgacattgacaataaaatcaacgaggtgaacgagatcgagaaactgctggtagttagcctgtaataa

SEQ ID NO: 37 - RNA, 1047 nt, Streptococcus sp.
  source 1..1047: mol_type = other RNA
atggccgaagttattagcggtagcgcagcaaccctgaatagcgcactggttaaaaatgttagcggtggcaaagcctatatcgacatctatgatgtgaaaaacggcaaaattgatccgctgaatctgattgttctgcctccgagcaattatagcgccaactattatatcaaacagggtggtcgcattttcaccaatgttaatcagctgcagacaccgggtacagcaaccattacctataacattctggatgaaaatggcaacccgtataccaaaagtgatggccagattgatattgttagcctggttaccaccgtttatgataccaccgaactgcgcaataacatcaacaaagttattgagaatgccaacgacccgaaatggtcagatgatagccgtaaagatgttctgagcaaaatcgaggtgatcaaaaacgatattgataacaacccgaaaacccagagcgatatcgacaacaaaattgtggaagtgaacgagctggaaaaactgctggttctgccggaatttagcaccattccgggttcagcagccacactgaataccagcattaccaaaaacattcagaatggcaacgcctacattgatctgtacgatgtaaaaaatggtctgatcgatccgcagaacctgatcgtgctgaatccgagcagctattcagccaattattatattaaacaaggcgcaaaatactatagcaacccgagcgaaattaccaccaccggtagcgccaccattacgtttaatatcctggacgaaaccggtaacccgcataaaaaagcagatggtcaaattgatatcgtgagcgttaacctgacgatttatgatagcacagccctgcgtaatcgtattgatgaagtgattaataacgcgaatgatcctaaatggtccgatggtagtcgtgatgaagtactgaccggtctggaaaaaatcaaaaaagacatcgacaataatccgaaaacgcagattgacattgacaataaaatcaacgaggtgaacgagatcgagaaactgctggtagttagcctgtaataa

SEQ ID NO: 38 - DNA, 1047 bp, Streptococcus sp.
  source 1..1047: mol_type = other DNA
atggccgaagttattagcggtagcgcagcaaccctgaatagcgcactggttaaaaatgttagcggtggcaaagcctatatcgacatctatgatgtgaaaaacggcaaaattgatccgctgaatctgattgttctgaccccgagcaattatagcgccaactattatatcaaacagggtggtcgtattttcaccagcgttaatcagctgcagacaccgggtacagcaaccattacctataacattctggatgaaaatggcaacccgtataccaaaagtgatggccagattgatattgttagcctggttaccaccgtttatgataccaccgaactgcgcaataacatcaacaaagttattgagaatgccaacgacccgaaatggtcagatgatagccgtaaagatgttctgagcaaaatcgaggtgatcaaaaacgatattgataacaacccgaaaacccagagcgatatcgacaacaaaattgtggaagtgaacgagctggaaaaactgctggttctgccggaatttagcaccattccgggttcagcagccacactgaataccagcattaccaaaaacattcagaatggcaacgcctacattgatctgtacgatgtaaaaaatggtctgatcgatccgcagaacctgatcgtgctgaatccgagcagctattcagccaattattatattaaacaaggcgcaaaatactatagcaacccgagcgaaattaccaccaccggtagcgccaccattacgtttaatatcctggacgaaaccggtaacccgcataaaaaagcagatggtcaaattgatatcgtgagcgttaacctgacgatttatgatagcacagccctgcgtaatcgtattgatgaagtgattaataacgcgaatgatcctaaatggtccgatggtagtcgtgatgaagtactgaccggtctggaaaaaatcaaaaaagacatcgacaataatccgaaaacgcagattgacattgacaataaaatcaacgaggtgaacgagatcgagaaactgctggtagttagcctgtaataa

SEQ ID NO: 39 - RNA, 1047 nt, Streptococcus sp.
  source 1..1047: mol_type = other RNA
atggccgaagttattagcggtagcgcagcaaccctgaatagcgcactggttaaaaatgttagcggtggcaaagcctatatcgacatctatgatgtgaaaaacggcaaaattgatccgctgaatctgattgttctgaccccgagcaattatagcgccaactattatatcaaacagggtggtcgtattttcaccagcgttaatcagctgcagacaccgggtacagcaaccattacctataacattctggatgaaaatggcaacccgtataccaaaagtgatggccagattgatattgttagcctggttaccaccgtttatgataccaccgaactgcgcaataacatcaacaaagttattgagaatgccaacgacccgaaatggtcagatgatagccgtaaagatgttctgagcaaaatcgaggtgatcaaaaacgatattgataacaacccgaaaacccagagcgatatcgacaacaaaattgtggaagtgaacgagctggaaaaactgctggttctgccggaatttagcaccattccgggttcagcagccacactgaataccagcattaccaaaaacattcagaatggcaacgcctacattgatctgtacgatgtaaaaaatggtctgatcgatccgcagaacctgatcgtgctgaatccgagcagctattcagccaattattatattaaacaaggcgcaaaatactatagcaacccgagcgaaattaccaccaccggtagcgccaccattacgtttaatatcctggacgaaaccggtaacccgcataaaaaagcagatggtcaaattgatatcgtgagcgttaacctgacgatttatgatagcacagccctgcgtaatcgtattgatgaagtgattaataacgcgaatgatcctaaatggtccgatggtagtcgtgatgaagtactgaccggtctggaaaaaatcaaaaaagacatcgacaataatccgaaaacgcagattgacattgacaataaaatcaacgaggtgaacgagatcgagaaactgctggtagttagcctgtaataa

SEQ ID NO: 40 - DNA, 1047 bp, Streptococcus sp.
  source 1..1047: mol_type = other DNA
atggccgaagtgatctccggctctgctgctaccctgaactctgccctggtcaagaatgtgtctggcggcaaggcctacatcgacatctacgacgtgaagaacggcaagatcgaccctctgaacctgatcgtgctgaccccttccaactactccgccaactactacatcaagcaaggcggcagaatcttcacctccgtgaaccagctgcagacccctggcaccgctaccatcacctacaacatcctggacgagaatggcaacccctacaccaagtccgacggccagatcgatatcgtgtccctggtcaccaccgtgtacgacaccaccgagctgcggaacaacatcaacaaagtgatcgagaacgccaacgatcccaagtggagcgacgactctagaaaggacgtgctgtccaagatcgaagtcatcaagaacgacatcgacaacaaccccaagacacagtccgacattgataacaagatcgtggaagtgaacgagctggaaaagctgctggtgctgcccgagttcagcacaatccctggatctgccgccacactgaacacctccatcaccaagaatatccagaacgggaacgcttacatcgacctgtatgatgtcaagaacgggctgatcgatccccagaatctgattgtgctcaacccctcctcctactctgctaattactatattaagcagggcgccaagtactactctaacccctccgagatcaccaccaccggctccgccaccatcacattcaatattctggatgagacaggcaaccctcacaagaaggctgacggacagattgacattgtgtctgtgaacctgaccatctacgattccaccgctctgcggaaccggatcgatgaagtgatcaacaacgctaatgaccctaagtggagtgacggctccagagatgaggtgctgaccggcctggaaaagatcaagaaggatatcgataacaatcctaaaactcagatcgatattgacaacaagatcaacgaagtcaacgagatcgagaagctcctggtcgtgtctctgtgatga

SEQ ID NO: 41 - RNA, 1047 nt, Streptococcus sp.
  source 1..1047: mol_type = other RNA
atggccgaagtgatctccggctctgctgctaccctgaactctgccctggtcaagaatgtgtctggcggcaaggcctacatcgacatctacgacgtgaagaacggcaagatcgaccctctgaacctgatcgtgctgaccccttccaactactccgccaactactacatcaagcaaggcggcagaatcttcacctccgtgaaccagctgcagacccctggcaccgctaccatcacctacaacatcctggacgagaatggcaacccctacaccaagtccgacggccagatcgatatcgtgtccctggtcaccaccgtgtacgacaccaccgagctgcggaacaacatcaacaaagtgatcgagaacgccaacgatcccaagtggagcgacgactctagaaaggacgtgctgtccaagatcgaagtcatcaagaacgacatcgacaacaaccccaagacacagtccgacattgataacaagatcgtggaagtgaacgagctggaaaagctgctggtgctgcccgagttcagcacaatccctggatctgccgccacactgaacacctccatcaccaagaatatccagaacgggaacgcttacatcgacctgtatgatgtcaagaacgggctgatcgatccccagaatctgattgtgctcaacccctcctcctactctgctaattactatattaagcagggcgccaagtactactctaacccctccgagatcaccaccaccggctccgccaccatcacattcaatattctggatgagacaggcaaccctcacaagaaggctgacggacagattgacattgtgtctgtgaacctgaccatctacgattccaccgctctgcggaaccggatcgatgaagtgatcaacaacgctaatgaccctaagtggagtgacggctccagagatgaggtgctgaccggcctggaaaagatcaagaaggatatcgataacaatcctaaaactcagatcgatattgacaacaagatcaacgaagtcaacgagatcgagaagctcctggtcgtgtctctgtgatga

SEQ ID NO: 42 - protein, 347 aa, Streptococcus sp.
MAEVISGSAATLNSALVKNVSGGKAYIDIYDVKNGKIDPLNLIVLTPSNYSANYYIKQGGRIFTSVNQLQTPGTATITYNILDENGNPYTKSDGQIDIVSLVTTVYDTTELRNNINKVIENANDPKWSDDSRKDVLSKIEVIKNDIDNNPKTQSDIDNKIVEVNELEKLLVLPEFSTIPGSAATLNTSITKNIQNGNAYIDLYDVKNGLIDPQNLIVLNPSSYSANYYIKQGAKYYSNPSEITTTGSATITFNILDETGNPHKKADGQIDIVSVNLTIYDSTALRNRIDEVINNANDPKWSDGSRDEVLTGLEKIKKDIDNNPKTQIDIDNKINEVNEIEKLLVVSL

SEQ ID NO: 43 - protein, 32 aa, Streptococcus sp.
GPLGSASVLIGISFLGGFTQGQFNISTDTVFA

SEQ ID NO: 44 - protein, 5 aa, Streptococcus sp.
GPLGS